European Patent Specification EP 3 655 021 B1, published March 22, 2023. Title: COMPOSITIONS AND METHODS FOR TREATING OR AMELIORATING SCLERODERMA-ASSOCIATED VASCULOPATHY. Applicant: Leadiant Biosciences Ltd. The sequence listing filed with the application follows.

SEQUENCE LISTING (4 sequences)

SEQ ID NO: 1 - protein, 356 aa, Mammalia
  MUTAGEN 74: Cys to Ser mutein
AQTPAFNKPKVELHVHLDGAIKPETILYYGRKRGIALPADTPEELQNIIGMDKPLSLPEFLAKFDYYMPAIAGSREAVKRIAYEFVEMKAKDGVVYVEVRYSPHLLANSKVEPIPWNQAEGDLTPDEVVSLVNQGLQEGERDFGVKVRSILCCMRHQPSWSSEVVELCKKYREQTVVAIDLAGDETIEGSSLFPGHVKAYAEAVKSGVHRTVHAGEVGSANVVKEAVDTLKTERLGHGYHTLEDTTLYNRLRQENMHFEVCPWSSYLTGAWKPDTEHPVVRFKNDQVNYSLNTDDPLIFKSTLDTDYQMTKNEMGFTEEEFKRLNINAAKSSFLPEDEKKELLDLLYKAYGMPSPA

SEQ ID NO: 2 - DNA, 1074 bp, Mammalia
atggctcagaccccggctttcaacaaaccgaaggtagaactgcacgtacacctggatggtgctatcaaaccggagactatcctgtactatggtcgtaagcgtggcatcgctctgccggctgacactccggaagaactgcagaacatcatcggcatggacaaaccgctgtctctgccggaattcctggctaaattcgactactacatgccggctatcgctggttctcgtgaagcagtcaaacgtatcgcttacgaattcgtagaaatgaaagctaaagatggtgtagtatacgttgaagttcgttactctccgcacctgctggcaaactctaaagttgaaccgatcccgtggaaccaggcagaaggcgatctgactccggatgaagtagtttctctggttaaccagggtctgcaggagggtgaacgcgatttcggcgtaaaagttcgttctatcctgtgctgcatgcgccaccagccgtcttggtcttctgaagttgttgaactgtgcaagaaataccgtgagcagaccgtagttgctatcgatctggcaggtgatgaaaccatcgaaggttcttctctgtttccgggtcacgtaaaggcttatgctgaagctgttaaatctggcgtacaccgtactgtacacgcaggtgaagttggttctgctaacgttgttaaagaagctgttgacaccctgaaaactgaacgcctgggtcacggctaccacaccctggaagacaccaccctgtacaaccgtctgcgtcaggaaaacatgcacttcgaagtttgtccgtggtcctcttacctgactggtgcttggaaaccggacaccgaacacccggttgttcgtttcaaaaacgaccaggtaaactactctctgaacactgacgatccgctgatcttcaaatctaccctggacaccgactaccagatgaccaaaaacgaaatgggtttcactgaagaagaattcaaacgtctgaacatcaacgctgctaagtcctcttttctgccggaagatgagaaaaaagaactgctggacctgctgtacaaggcatacggtatgccgtctccggcttaa

SEQ ID NO: 3 - protein, 362 aa, Homo sapiens
  (74)...(74) Cys to Ser mutein
  MUTAGEN 74: Cys to Ser mutein
AQTPAFDKPKVELHVHLDGSIKPETILYYGRRRGIALPANTAEGLLNVIGMDKPLTLPDFLAKFDYYMPAIAGSREAIKRIAYEFVEMKAKEGVVYVEVRYSPHLLANSKVEPIPWNQAEGDLTPDEVVALVGQGLQEGERDFGVKARSILCCMRHQPNWSPKVVELCKKYQQQTVVAIDLAGDETIPGSSLLPGHVQAYQEAVKSGIHRTVHAGEVGSAEVVKEAVDILKTERLGHGYHTLEDQALYNRLRQENMHFEICPWSSYLTGAWKPDTEHAVIRLKNDQANYSLNTDDPLIFKSTLDTDYQMTKRDMGFTEEEFKRLNINAAKSSFLPEDEKRELLDLLYKAYGMPPSASAGQNL

SEQ ID NO: 4 - DNA, 1089 bp, Homo sapiens
atggctcagacacccgcatttgataaaccgaaagtggaactgcatgtccacctggatggtagcatcaaaccggaaactatcttatattacggtcggcgtcgtggtattgcgttgccggcaaacacggctgaaggtttgctgaacgtgatcggcatggacaaaccgctgaccttgccggattttttggcgaaatttgattattatatgccggcgattgctggttcccgcgaggcaatcaaacgcatcgcgtatgagtttgttgaaatgaaagcgaaagaaggcgttgtgtatgttgaggtccgttacagtccgcatctgctggctaacagcaaggtagaacctatcccctggaaccaagctgaaggcgatctgacgccggatgaagtggttgctctggtgggtcagggtttacaggagggggagcgcgattttggcgttaaagctcgctctattttatgttgcatgcgccatcagcccaattggtccccgaaagtggttgaactttgtaaaaagtaccaacaacagaccgttgtcgcgattgatttggcaggcgatgaaacaattccaggcagctccctgttgccagggcacgtgcaagcgtaccaagaagcagtgaaaagcggcatccaccggactgtccacgccggcgaggtcggtagcgccgaggttgtgaaagaagccgtggacatcctgaaaaccgagcggctgggccatgggtaccacacactggaggatcaggcattatataaccgcttacgccaggaaaatatgcatttcgaaatttgtccgtggagtagttacttaactggcgcgtggaaaccggataccgaacatgcggttatccgcttaaagaatgatcaagcaaattacagtctgaatacagatgatcccctgattttcaagtctaccctggacacagattatcagatgacgaagcgggatatgggatttacggaagaagaatttaagcgtctcaatatcaatgcggcgaaatcttcatttctgccggaagatgagaaacgtgagttgctggatcttctgtacaaggcctacggtatgccgccgagcgcatcggccgggcagaacctg